European Patent Specification EP 4 135 745 B1, published May 7, 2025. Title: sCD83 for Wound Healing, Hair Growth, and Skin and Hair Care. Applicant: Friedrich-Alexander-Universitaet Erlangen-Nuernberg. The sequence listing filed with the application follows.

SEQUENCE LISTING (50 sequences)

SEQ ID NO: 1 - DNA, 618 bp, Homo sapiens
  CDS (1)..(615)
atgtcgcgcggcctccagcttctgctcctgagctgcgcctacagcctggctcccgcgacgccggaggtgaaggtggcttgctccgaagatgtggacttgccctgcaccgccccctgggatccgcaggttccctacacggtctcctgggtcaagttattggagggtggtgaagagaggatggagacaccccaggaagaccacctcaggggacagcactatcatcagaaggggcaaaatggttctttcgacgcccccaatgaaaggccctattccctgaagatccgaaacactaccagctgcaactcggggacatacaggtgcactctgcaggacccggatgggcagagaaacctaagtggcaaggtgatcttgagagtgacaggatgccctgcacagcgtaaagaagagacttttaagaaatacagagcggagattgtcctgctgctggctctggttattttctacttaacactcatcattttcacttgtaagtttgcacggctacagagtatcttcccagatttttctaaagctggcatggaacgagcttttctcccagttacctccccaaataagcatttagggctagtgactcctcacaagacagaactggtatga

SEQ ID NO: 2 - protein, 205 aa, Homo sapiens
MSRGLQLLLLSCAYSLAPATPEVKVACSEDVDLPCTAPWDPQVPYTVSWVKLLEGGEERMETPQEDHLRGQHYHQKGQNGSFDAPNERPYSLKIRNTTSCNSGTYRCTLQDPDGQRNLSGKVILRVTGCPAQRKEETFKKYRAEIVLLLALVIFYLTLIIFTCKFARLQSIFPDFSKAGMERAFLPVTSPNKHLGLVTPHKTELV

SEQ ID NO: 3 - DNA, 2051 bp, Mus musculus
  CDS (14)..(601)
gcgctccagccgcatgtcgcaaggcctccagctcctgtttctaggctgcgcctgcagcctggcacccgcgatggcgatgcgggaggtgacggtggcttgctccgagaccgccgacttgccttgcacagcgccctgggacccgcagctctcctatgcagtgtcctgggccaaggtctccgagagtggcactgagagtgtggagctcccggagagcaagcaaaacagctccttcgaggcccccaggagaagggcctattccctgacgatccaaaacactaccatctgcagctcgggcacctacaggtgtgccctgcaggagctcggagggcagcgcaacttgagcggcaccgtggttctgaaggtgacaggatgccccaaggaagctacagagtcaactttcaggaagtacagggcagaagctgtgttgctcttctctctggttgttttctacctgacactcatcattttcacctgcaaatttgcacgactacaaagcattttcccagatatttctaaacctggtacggaacaagcttttcttccagtcacctccccaagcaaacatttggggccagtgacccttcctaagacagaaacggtatgagtaggatctccactggtttttacaaagccaagggcacatcagatcagtgtgcctgaatgccacccggacaagagaagaatgagctccatcctcagatggcaacctttctttgaagtccttcacctgacagtgggctccacactactccctgacacagggtcttgagcaccatcatatgatcacgaagcatggagtatcaccgcttctctgtggctgtcagcttaatgtttcatgtggctatctggtcaacctcgtgagtgcttttcagtcatctacaagctatggtgagatgcaggtgaagcagggtcatgggaaatttgaacactctgagctggccctgtgacagactcctgaggacagctgtcctctcctacatctgggatacatctctttgaatttgtcctgtttcgttgcaccagcccagatgtctcacatctggcggaaattgacaggccaagctgtgagccagtgggaaatatttagcaaataatttcccagtgcgaaggtcctgctattagtaaggagtattatgtgtacatagaaatgagaggtcagtgaactattccccagcagggccttttcatctggaaaagacatccacaaaagcagcaatacagagggatgccacatttatttttttaatcttcatgtacttgtcaaagaagaatttttcatgttttttcaaagaagtgtgtttctttccttttttaaaatatgaaggtctagttacatagcattgctagctgacaagcagcctgagagaagatggagaatgttcctcaaaatagggacagcaagctagaagcactgtacagtgccctgctgggaagggcagacaatggactgagaaaccagaagtctggccacaagattgtctgtatgattctggacgagtcacttgtggttttcactctctggttagtaaaccagatagtttagtctgggttgaatacaatggatgtgaagttgcttggggaaagctgaatgtagtgaatacattggcaactctactgggctgttaccttgttgatatcctagagttctggagctgagcgaatgcctgtcatatctcagcttgcccatcaatccaaacacaggaggctacaaaaaggacatgagcatggtcttctgtgtgaactcctcctgagaaacgtggagactggctcagcgctttgcgcttgaaggactaatcacaagttcttgaagatatggacctaggggagctattgcgccacgacaggaggaagttctcagatgttgcattgatgtaacattgttgcatttctttaatgagctgggctccttcctcatttgcttcccaaagagattttgtcccactaatggtgtgcccatcacccacactatgaaagtaaaagggatgctgagcagatacagcgtgcttacctctcagccatgactttcatgctattaaaagaatgcatgtgaa

SEQ ID NO: 4 - protein, 196 aa, Mus musculus
MSQGLQLLFLGCACSLAPAMAMREVTVACSETADLPCTAPWDPQLSYAVSWAKVSESGTESVELPESKQNSSFEAPRRRAYSLTIQNTTICSSGTYRCALQELGGQRNLSGTVVLKVTGCPKEATESTFRKYRAEAVLLFSLVVFYLTLIIFTCKFARLQSIFPDISKPGTEQAFLPVTSPSKHLGPVTLPKTETV

SEQ ID NO: 5 - DNA, 31 bp, Artificial Sequence
  Description of Artificial Sequence: primer for CD83ext
tcccccgggaacgccggaggtgaaggtggct

SEQ ID NO: 6 - DNA, 31 bp, Artificial Sequence
  Description of Artificial Sequence: primer for CD83ext
aattagaattctcaaatctccgctctgtatt

SEQ ID NO: 7 - DNA, 435 bp, Artificial Sequence
  Description of Artificial Sequence: partial sequence of pGEX2ThCD83ext
  CDS (1)..(417)
  mat_peptide (28)..(417)
cctccaaaatcggatctggttccgcgtggatccccgggaacgccggaggtgaaggtggcttgctccgaagatgtggacttgccctgcaccgccccctgggatccgcaggttccctacacggtctcctgggtcaagttattggagggtggtgaagagaggatggagacaccccaggaagaccacctcaggggacagcactatcatcagaaggggcaaaatggttctttcgacgcccccaatgaaaggccctattccctgaagatccgaaacactaccagctgcaactcggggacatacaggtgcactctgcaggacccggatgggcagagaaacctaagtggcaaggtgatcttgagagtgacaggatgccctgcacagcgtaaagaagagacttttaagaaatacagagcggagatttgagaattcatcgtgact

SEQ ID NO: 8 - protein, 139 aa, Artificial Sequence
  Description of Artificial Sequence: partial sequence of pGEX2ThCD83ext
PPKSDLVPRGSPGTPEVKVACSEDVDLPCTAPWDPQVPYTVSWVKLLEGGEERMETPQEDHLRGQHYHQKGQNGSFDAPNERPYSLKIRNTTSCNSGTYRCTLQDPDGQRNLSGKVILRVTGCPAQRKEETFKKYRAEI

SEQ ID NO: 9 - DNA, 435 bp, Artificial Sequence
  Description of Artificial Sequence: partial sequence of pGEX2ThCD83ext_mut129_CtoS
  CDS (1)..(417)
  mat_peptide (28)..(417)
cctccaaaatcggatctggttccgcgtggatccccgggaacgccggaggtgaaggtggcttgctccgaagatgtggacttgccctgcaccgccccctgggatccgcaggttccctacacggtctcctgggtcaagttattggagggtggtgaagagaggatggagacaccccaggaagaccacctcaggggacagcactatcatcagaaggggcaaaatggttctttcgacgcccccaatgaaaggccctattccctgaagatccgaaacactaccagctgcaactcggggacatacaggtgcactctgcaggacccggatgggcagagaaacctaagtggcaaggtgatcttgagagtgacaggatcccctgcacagcgtaaagaagagacttttaagaaatacagagcggagatttgagaattcatcgtgact

SEQ ID NO: 10 - protein, 139 aa, Artificial Sequence
  Description of Artificial Sequence: partial sequence of pGEX2ThCD83ext_mut129_CtoS
PPKSDLVPRGSPGTPEVKVACSEDVDLPCTAPWDPQVPYTVSWVKLLEGGEERMETPQEDHLRGQHYHQKGQNGSFDAPNERPYSLKIRNTTSCNSGTYRCTLQDPDGQRNLSGKVILRVTGSPAQRKEETFKKYRAEI

SEQ ID NO: 11 - DNA, 402 bp, Arteficial Sequence
  Description of Artificial Sequence: N6HIS-sCD83
  CDS (1)..(402)
taccatcatcaccaccaccatacgccggaggtgaaggtggcttgctccgaagatgtggacttgccctgcaccgccccctgggatccgcaggttccctacacggtctcctgggtcaagttattggagggtggtgaagagaggatggagacaccccaggaagaccacctcaggggacagcactatcatcagaaggggcaaaatggttctttcgacgcccccaatgaaaggccctattccctgaagatccgaaacactaccagctgcaactcggggacatacaggtgcactctgcaggacccggatgggcagagaaacctaagtggcaaggtgatcttgagagtgacaggatgccctgcacagcgtaaagaagagacttttaagaaatacagagcggagatttga

SEQ ID NO: 12 - protein, 133 aa, Arteficial Sequence
  Description of Artificial Sequence: N6HIS-sCD83
YHHHHHHTPEVKVACSEDVDLPCTAPWDPQVPYTVSWVKLLEGGEERMETPQEDHLRGQHYHQKGQNGSFDAPNERPYSLKIRNTTSCNSGTYRCTLQDPDGQRNLSGKVILRVTGCPAQRKEETFKKYRAEI

SEQ ID NO: 13 - DNA, 20 bp, Mus musculus
tccagaaggccctcagacta

SEQ ID NO: 14 - DNA, 20 bp, Mus musculus
agcatcttctcgaccctgaa

SEQ ID NO: 15 - DNA, 21 bp, Mus musculus
cccaggaaagacagcaacctt

SEQ ID NO: 16 - DNA, 21 bp, Mus musculus
ccttgcctttctcatccagga

SEQ ID NO: 17 - DNA, 20 bp, Mus musculus
cagccatttgcacacctcac

SEQ ID NO: 18 - DNA, 20 bp, Mus musculus
cccgatgtttcatgatgccg

SEQ ID NO: 19 - DNA, 19 bp, Mus musculus
gtgatcggtccccaaaggg

SEQ ID NO: 20 - DNA, 19 bp, Mus musculus
ccagctgctcctccacttg

SEQ ID NO: 21 - DNA, 21 bp, Mus musculus
tgccaccttttgacagtgatg

SEQ ID NO: 22 - DNA, 20 bp, Mus musculus
atgtgctgctgcgagatttg

SEQ ID NO: 23 - DNA, 20 bp, Mus musculus
gctgaacccttacgccaaga

SEQ ID NO: 24 - DNA, 20 bp, Mus musculus
tctcggatttggttgccagt

SEQ ID NO: 25 - DNA, 20 bp, Mus musculus
gctttgcagctcttcctcat

SEQ ID NO: 26 - DNA, 20 bp, Mus musculus
gtcaccatccttttgccagt

SEQ ID NO: 27 - DNA, 20 bp, Mus musculus
ccaagccttatcggaaatga

SEQ ID NO: 28 - DNA, 20 bp, Mus musculus
ttttcacaggggagaaatcg

SEQ ID NO: 29 - DNA, 22 bp, Mus musculus
tggagcaacatgtggaactcta

SEQ ID NO: 30 - DNA, 21 bp, Mus musculus
agacagccactcaggcgtatc

SEQ ID NO: 31 - DNA, 20 bp, Mus musculus
gctttgcagctcttcctcat

SEQ ID NO: 32 - DNA, 20 bp, Mus musculus
gtcaccatccttttgccagt

SEQ ID NO: 33 - DNA, 22 bp, Mus musculus
acaaagccagagtccttcagag

SEQ ID NO: 34 - DNA, 22 bp, Mus musculus
gagcattggaaattggggtagg

SEQ ID NO: 35 - DNA, 20 bp, Mus musculus
gctgtacaagcagtggcaaa

SEQ ID NO: 36 - DNA, 20 bp, Mus musculus
ccccaaagatagcatctgga

SEQ ID NO: 37 - DNA, 21 bp, Mus musculus
gagagctacaagaggatcacc

SEQ ID NO: 38 - DNA, 21 bp, Mus musculus
gatctcatttggttccgatcc

SEQ ID NO: 39 - DNA, 20 bp, Mus musculus
gacttgcgtgactatgaagc

SEQ ID NO: 40 - DNA, 22 bp, Mus musculus
tgaatatctgacggttctgagg

SEQ ID NO: 41 - DNA, 23 bp, Mus musculus
acattggctcacttccagaaaca

SEQ ID NO: 42 - DNA, 22 bp, Mus musculus
ggttggaaccggcatctttatc

SEQ ID NO: 43 - DNA, 21 bp, Mus musculus
ggccttttacctttcacggtg

SEQ ID NO: 44 - DNA, 21 bp, Mus musculus
tacggcattgtggcttctcaa

SEQ ID NO: 45 - DNA, 758 bp, Artificial Sequence
  Description of Artificial Sequence: pPIC9K fragment
tccaaacgatgagatttccttcaatttttactgcagttttattcgcagcatcctccgcattagctgctccagtcaacactacaacagaagatgaaacggcacaaattccggctgaagctgtcatcggttactcagatttagaaggggatttcgatgttgctgttttgccattttccaacagcacaaataacgggttattgtttataaatactactattgccagcattgctgctaaagaagaaggggtatctctcgagaaaagagaggctgaagcttaccatcatcaccaccaccatacgccggaggtgaaggtggcttgctccgaagatgtggacttgccctgcaccgccccctgggatccgcaggttccctacacggtctcctgggtcaagttattggagggtggtgaagagaggatggagacaccccaggaagaccacctcaggggacagcactatcatcagaaggggcaaaatggttctttcgacgcccccaatgaaaggccctattccctgaagatccgaaacactaccagctgcaactcggggacatacaggtgcactctgcaggacccggatgggcagagaaacctaagtggcaaggtgatcttgagagtgacaggatgccctgcacagcgtaaagaagagacttttaagaaatacagagcggagatttgagtagaattccctagggcggccgcgaattaattcgccttagacatgactgttcctcagttcaagttgggcacttacgagaag

SEQ ID NO: 46 - DNA, 12 bp, Arteficial Sequence
  Description of Artificial Sequence: Glu-Ala-Glu-Ala-repeats
gaggctgaagct

SEQ ID NO: 47 - DNA, 18 bp, Arteficial Sequence
  Description of Artificial Sequence: 6HIS
catcatcaccaccaccat

SEQ ID NO: 48 - DNA, 378 bp, Homo sapiens
acgccggaggtgaaggtggcttgctccgaagatgtggacttgccctgcaccgccccctgggatccgcaggttccctacacggtctcctgggtcaagttattggagggtggtgaagagaggatggagacaccccaggaagaccacctcaggggacagcactatcatcagaaggggcaaaatggttctttcgacgcccccaatgaaaggccctattccctgaagatccgaaacactaccagctgcaactcggggacatacaggtgcactctgcaggacccggatgggcagagaaacctaagtggcaaggtgatcttgagagtgacaggatgccctgcacagcgtaaagaagagacttttaagaaatacagagcggagatt

SEQ ID NO: 49 - DNA, 681 bp, Homo sapiens
  CDS (1)..(681)
gacaaaactcacacatgcccaccgtgcccagcacctgaactcctggggggaccgtcagtcttcctcttccccccaaaacccaaggacaccctcatgatctcccggacccctgaggtcacatgcgtggtggtggacgtgagccacgaagaccctgaggtcaagttcaactggtacgtggacggcgtggaggtgcataatgccaagacaaagccgcgggaggagcagtacaacagcacgtaccgtgtggtcagcgtcctcaccgtcctgcaccaggactggctgaatggcaaggagtacaagtgcaaggtctccaacaaagccctcccagcccccatcgagaaaaccatctccaaagccaaagggcagccccgagaaccacaggtgtacaccctgcccccatcccgggaggagatgaccaagaaccaggtcagcctgacctgcctggtcaaaggcttctatcccagcgacatcgccgtggagtgggagagcaatgggcagccggagaacaactacaagaccacgcctcccgtgctggactccgacggctccttcttcctctacagcaagctcaccgtggacaagagcaggtggcagcaggggaacgtcttctcatgctccgtgatgcacgaggctctgcacaaccactacacgcagaagagcctctccctgtctccgggtaaa

SEQ ID NO: 50 - protein, 227 aa, Homo sapiens
DKTHTCPPCPAPELLGGPSVFLFPPKPKDTLMISRTPEVTCVVVDVSHEDPEVKFNWYVDGVEVHNAKTKPREEQYNSTYRVVSVLTVLHQDWLNGKEYKCKVSNKALPAPIEKTISKAKGQPREPQVYTLPPSREEMTKNQVSLTCLVKGFYPSDIAVEWESNGQPENNYKTTPPVLDSDGSFFLYSKLTVDKSRWQQGNVFSCSVMHEALHNHYTQKSLSLSPGK